European Patent Specification EP 4 017 976 B1, published July 2, 2025. Title: Coiled-coil mediated tethering of CRISPR/CAS and exonucleases for enhanced genome editing. Applicant: National Institute of Chemistry. The sequence listing filed with the application follows.

SEQUENCE LISTING (29 sequences)

SEQ ID NO: 1 - DNA, 4308 bp, Artificial Sequence
  Cas9-P4
atggccccaaagaagaagcggaaggtcggtatccacggagtcccagcagccgacaagaagtacagcatcggcctggacatcggcaccaactctgtgggctgggccgtgatcaccgacgagtacaaggtgcccagcaagaaattcaaggtgctgggcaacaccgaccggcacagcatcaagaagaacctgatcggagccctgctgttcgacagcggcgaaacagccgaggccacccggctgaagagaaccgccagaagaagatacaccagacggaagaaccggatctgctatctgcaagagatcttcagcaacgagatggccaaggtggacgacagcttcttccacagactggaagagtccttcctggtggaagaggataagaagcacgagcggcaccccatcttcggcaacatcgtggacgaggtggcctaccacgagaagtaccccaccatctaccacctgagaaagaaactggtggacagcaccgacaaggccgacctgcggctgatctatctggccctggcccacatgatcaagttccggggccacttcctgatcgagggcgacctgaaccccgacaacagcgacgtggacaagctgttcatccagctggtgcagacctacaaccagctgttcgaggaaaaccccatcaacgccagcggcgtggacgccaaggccatcctgtctgccagactgagcaagagcagacggctggaaaatctgatcgcccagctgcccggcgagaagaagaatggcctgttcggaaacctgattgccctgagcctgggcctgacccccaacttcaagagcaacttcgacctggccgaggatgccaaactgcagctgagcaaggacacctacgacgacgacctggacaacctgctggcccagatcggcgaccagtacgccgacctgtttctggccgccaagaacctgtccgacgccatcctgctgagcgacatcctgagagtgaacaccgagatcaccaaggcccccctgagcgcctctatgatcaagagatacgacgagcaccaccaggacctgaccctgctgaaagctctcgtgcggcagcagctgcctgagaagtacaaagagattttcttcgaccagagcaagaacggctacgccggctacattgacggcggagccagccaggaagagttctacaagttcatcaagcccatcctggaaaagatggacggcaccgaggaactgctcgtgaagctgaacagagaggacctgctgcggaagcagcggaccttcgacaacggcagcatcccccaccagatccacctgggagagctgcacgccattctgcggcggcaggaagatttttacccattcctgaaggacaaccgggaaaagatcgagaagatcctgaccttccgcatcccctactacgtgggccctctggccaggggaaacagcagattcgcctggatgaccagaaagagcgaggaaaccatcaccccctggaacttcgaggaagtggtggacaagggcgcttccgcccagagcttcatcgagcggatgaccaacttcgataagaacctgcccaacgagaaggtgctgcccaagcacagcctgctgtacgagtacttcaccgtgtataacgagctgaccaaagtgaaatacgtgaccgagggaatgagaaagcccgccttcctgagcggcgagcagaaaaaggccatcgtggacctgctgttcaagaccaaccggaaagtgaccgtgaagcagctgaaagaggactacttcaagaaaatcgagtgcttcgactccgtggaaatctccggcgtggaagatcggttcaacgcctccctgggcacataccacgatctgctgaaaattatcaaggacaaggacttcctggacaatgaggaaaacgaggacattctggaagatatcgtgctgaccctgacactgtttgaggacagagagatgatcgaggaacggctgaaaacctatgcccacctgttcgacgacaaagtgatgaagcagctgaagcggcggagatacaccggctggggcaggctgagccggaagctgatcaacggcatccgggacaagcagtccggcaagacaatcctggatttcctgaagtccgacggcttcgccaacagaaacttcatgcagctgatccacgacgacagcctgacctttaaagaggacatccagaaagcccaggtgtccggccagggcgatagcctgcacgagcacattgccaatctggccggcagccccgccattaagaagggcatcctgcagacagtgaaggtggtggacgagctcgtgaaagtgatgggccggcacaagcccgagaacatcgtgatcgaaatggccagagagaaccagaccacccagaagggacagaagaacagccgcgagagaatgaagcggatcgaagagggcatcaaagagctgggcagccagatcctgaaagaacaccccgtggaaaacacccagctgcagaacgagaagctgtacctgtactacctgcagaatgggcgggatatgtacgtggaccaggaactggacatcaaccggctgtccgactacgatgtggaccatatcgtgcctcagagctttctgaaggacgactccatcgacaacaaggtgctgaccagaagcgacaagaaccggggcaagagcgacaacgtgccctccgaagaggtcgtgaagaagatgaagaactactggcggcagctgctgaacgccaagctgattacccagagaaagttcgacaatctgaccaaggccgagagaggcggcctgagcgaactggataaggccggcttcatcaagagacagctggtggaaacccggcagatcacaaagcacgtggcacagatcctggactcccggatgaacactaagtacgacgagaatgacaagctgatccgggaagtgaaagtgatcaccctgaagtccaagctggtgtccgatttccggaaggatttccagttttacaaagtgcgcgagatcaacaactaccaccacgcccacgacgcctacctgaacgccgtcgtgggaaccgccctgatcaaaaagtaccctaagctggaaagcgagttcgtgtacggcgactacaaggtgtacgacgtgcggaagatgatcgccaagagcgagcaggaaatcggcaaggctaccgccaagtacttcttctacagcaacatcatgaactttttcaagaccgagattaccctggccaacggcgagatccggaagcggcctctgatcgagacaaacggcgaaaccggggagatcgtgtgggataagggccgggattttgccaccgtgcggaaagtgctgagcatgccccaagtgaatatcgtgaaaaagaccgaggtgcagacaggcggcttcagcaaagagtctatcctgcccaagaggaacagcgataagctgatcgccagaaagaaggactgggaccctaagaagtacggcggcttcgacagccccaccgtggcctattctgtgctggtggtggccaaagtggaaaagggcaagtccaagaaactgaagagtgtgaaagagctgctggggatcaccatcatggaaagaagcagcttcgagaagaatcccatcgactttctggaagccaagggctacaaagaagtgaaaaaggacctgatcatcaagctgcctaagtactccctgttcgagctggaaaacggccggaagagaatgctggcctctgccggcgaactgcagaagggaaacgaactggccctgccctccaaatatgtgaacttcctgtacctggccagccactatgagaagctgaagggctcccccgaggataatgagcagaaacagctgtttgtggaacagcacaagcactacctggacgagatcatcgagcagatcagcgagttctccaagagagtgatcctggccgacgctaatctggacaaagtgctgtccgcctacaacaagcaccgggataagcccatcagagagcaggccgagaatatcatccacctgtttaccctgaccaatctgggagcccctgccgccttcaagtactttgacaccaccatcgaccggaagaggtacaccagcaccaaagaggtgctggacgccaccctgatccaccagagcatcaccggcctgtacgagacacggatcgacctgtctcagctgggaggcgacgatccaaaaaagaagagaaaggtaggcggctctggcggcggctccggaggctctagcccggaagataaaattgctcagctgaaacaaaaaatccaagcgctgaaacaggaaaaccagcagctggaagaggaaaacgccgcactggaatatggttaa

SEQ ID NO: 2 - DNA, 4308 bp, Artificial Sequence
  Cas9-P3
atggccccaaagaagaagcggaaggtcggtatccacggagtcccagcagccgacaagaagtacagcatcggcctggacatcggcaccaactctgtgggctgggccgtgatcaccgacgagtacaaggtgcccagcaagaaattcaaggtgctgggcaacaccgaccggcacagcatcaagaagaacctgatcggagccctgctgttcgacagcggcgaaacagccgaggccacccggctgaagagaaccgccagaagaagatacaccagacggaagaaccggatctgctatctgcaagagatcttcagcaacgagatggccaaggtggacgacagcttcttccacagactggaagagtccttcctggtggaagaggataagaagcacgagcggcaccccatcttcggcaacatcgtggacgaggtggcctaccacgagaagtaccccaccatctaccacctgagaaagaaactggtggacagcaccgacaaggccgacctgcggctgatctatctggccctggcccacatgatcaagttccggggccacttcctgatcgagggcgacctgaaccccgacaacagcgacgtggacaagctgttcatccagctggtgcagacctacaaccagctgttcgaggaaaaccccatcaacgccagcggcgtggacgccaaggccatcctgtctgccagactgagcaagagcagacggctggaaaatctgatcgcccagctgcccggcgagaagaagaatggcctgttcggaaacctgattgccctgagcctgggcctgacccccaacttcaagagcaacttcgacctggccgaggatgccaaactgcagctgagcaaggacacctacgacgacgacctggacaacctgctggcccagatcggcgaccagtacgccgacctgtttctggccgccaagaacctgtccgacgccatcctgctgagcgacatcctgagagtgaacaccgagatcaccaaggcccccctgagcgcctctatgatcaagagatacgacgagcaccaccaggacctgaccctgctgaaagctctcgtgcggcagcagctgcctgagaagtacaaagagattttcttcgaccagagcaagaacggctacgccggctacattgacggcggagccagccaggaagagttctacaagttcatcaagcccatcctggaaaagatggacggcaccgaggaactgctcgtgaagctgaacagagaggacctgctgcggaagcagcggaccttcgacaacggcagcatcccccaccagatccacctgggagagctgcacgccattctgcggcggcaggaagatttttacccattcctgaaggacaaccgggaaaagatcgagaagatcctgaccttccgcatcccctactacgtgggccctctggccaggggaaacagcagattcgcctggatgaccagaaagagcgaggaaaccatcaccccctggaacttcgaggaagtggtggacaagggcgcttccgcccagagcttcatcgagcggatgaccaacttcgataagaacctgcccaacgagaaggtgctgcccaagcacagcctgctgtacgagtacttcaccgtgtataacgagctgaccaaagtgaaatacgtgaccgagggaatgagaaagcccgccttcctgagcggcgagcagaaaaaggccatcgtggacctgctgttcaagaccaaccggaaagtgaccgtgaagcagctgaaagaggactacttcaagaaaatcgagtgcttcgactccgtggaaatctccggcgtggaagatcggttcaacgcctccctgggcacataccacgatctgctgaaaattatcaaggacaaggacttcctggacaatgaggaaaacgaggacattctggaagatatcgtgctgaccctgacactgtttgaggacagagagatgatcgaggaacggctgaaaacctatgcccacctgttcgacgacaaagtgatgaagcagctgaagcggcggagatacaccggctggggcaggctgagccggaagctgatcaacggcatccgggacaagcagtccggcaagacaatcctggatttcctgaagtccgacggcttcgccaacagaaacttcatgcagctgatccacgacgacagcctgacctttaaagaggacatccagaaagcccaggtgtccggccagggcgatagcctgcacgagcacattgccaatctggccggcagccccgccattaagaagggcatcctgcagacagtgaaggtggtggacgagctcgtgaaagtgatgggccggcacaagcccgagaacatcgtgatcgaaatggccagagagaaccagaccacccagaagggacagaagaacagccgcgagagaatgaagcggatcgaagagggcatcaaagagctgggcagccagatcctgaaagaacaccccgtggaaaacacccagctgcagaacgagaagctgtacctgtactacctgcagaatgggcgggatatgtacgtggaccaggaactggacatcaaccggctgtccgactacgatgtggaccatatcgtgcctcagagctttctgaaggacgactccatcgacaacaaggtgctgaccagaagcgacaagaaccggggcaagagcgacaacgtgccctccgaagaggtcgtgaagaagatgaagaactactggcggcagctgctgaacgccaagctgattacccagagaaagttcgacaatctgaccaaggccgagagaggcggcctgagcgaactggataaggccggcttcatcaagagacagctggtggaaacccggcagatcacaaagcacgtggcacagatcctggactcccggatgaacactaagtacgacgagaatgacaagctgatccgggaagtgaaagtgatcaccctgaagtccaagctggtgtccgatttccggaaggatttccagttttacaaagtgcgcgagatcaacaactaccaccacgcccacgacgcctacctgaacgccgtcgtgggaaccgccctgatcaaaaagtaccctaagctggaaagcgagttcgtgtacggcgactacaaggtgtacgacgtgcggaagatgatcgccaagagcgagcaggaaatcggcaaggctaccgccaagtacttcttctacagcaacatcatgaactttttcaagaccgagattaccctggccaacggcgagatccggaagcggcctctgatcgagacaaacggcgaaaccggggagatcgtgtgggataagggccgggattttgccaccgtgcggaaagtgctgagcatgccccaagtgaatatcgtgaaaaagaccgaggtgcagacaggcggcttcagcaaagagtctatcctgcccaagaggaacagcgataagctgatcgccagaaagaaggactgggaccctaagaagtacggcggcttcgacagccccaccgtggcctattctgtgctggtggtggccaaagtggaaaagggcaagtccaagaaactgaagagtgtgaaagagctgctggggatcaccatcatggaaagaagcagcttcgagaagaatcccatcgactttctggaagccaagggctacaaagaagtgaaaaaggacctgatcatcaagctgcctaagtactccctgttcgagctggaaaacggccggaagagaatgctggcctctgccggcgaactgcagaagggaaacgaactggccctgccctccaaatatgtgaacttcctgtacctggccagccactatgagaagctgaagggctcccccgaggataatgagcagaaacagctgtttgtggaacagcacaagcactacctggacgagatcatcgagcagatcagcgagttctccaagagagtgatcctggccgacgctaatctggacaaagtgctgtccgcctacaacaagcaccgggataagcccatcagagagcaggccgagaatatcatccacctgtttaccctgaccaatctgggagcccctgccgccttcaagtactttgacaccaccatcgaccggaagaggtacaccagcaccaaagaggtgctggacgccaccctgatccaccagagcatcaccggcctgtacgagacacggatcgacctgtctcagctgggaggcgacgatccaaaaaagaagagaaaggtaggcggctctggcggcggctccggaggctcttccccggaagatgagatccagcaactggaagaagaaatcgctcagctggaacagaaaaacgcagcgctgaaagagaaaaaccaggcgctgaaatacggttaa

SEQ ID NO: 3 - DNA, 4293 bp, Artificial Sequence
  Cas9-N5
atggccccaaagaagaagcggaaggtcggtatccacggagtcccagcagccgacaagaagtacagcatcggcctggacatcggcaccaactctgtgggctgggccgtgatcaccgacgagtacaaggtgcccagcaagaaattcaaggtgctgggcaacaccgaccggcacagcatcaagaagaacctgatcggagccctgctgttcgacagcggcgaaacagccgaggccacccggctgaagagaaccgccagaagaagatacaccagacggaagaaccggatctgctatctgcaagagatcttcagcaacgagatggccaaggtggacgacagcttcttccacagactggaagagtccttcctggtggaagaggataagaagcacgagcggcaccccatcttcggcaacatcgtggacgaggtggcctaccacgagaagtaccccaccatctaccacctgagaaagaaactggtggacagcaccgacaaggccgacctgcggctgatctatctggccctggcccacatgatcaagttccggggccacttcctgatcgagggcgacctgaaccccgacaacagcgacgtggacaagctgttcatccagctggtgcagacctacaaccagctgttcgaggaaaaccccatcaacgccagcggcgtggacgccaaggccatcctgtctgccagactgagcaagagcagacggctggaaaatctgatcgcccagctgcccggcgagaagaagaatggcctgttcggaaacctgattgccctgagcctgggcctgacccccaacttcaagagcaacttcgacctggccgaggatgccaaactgcagctgagcaaggacacctacgacgacgacctggacaacctgctggcccagatcggcgaccagtacgccgacctgtttctggccgccaagaacctgtccgacgccatcctgctgagcgacatcctgagagtgaacaccgagatcaccaaggcccccctgagcgcctctatgatcaagagatacgacgagcaccaccaggacctgaccctgctgaaagctctcgtgcggcagcagctgcctgagaagtacaaagagattttcttcgaccagagcaagaacggctacgccggctacattgacggcggagccagccaggaagagttctacaagttcatcaagcccatcctggaaaagatggacggcaccgaggaactgctcgtgaagctgaacagagaggacctgctgcggaagcagcggaccttcgacaacggcagcatcccccaccagatccacctgggagagctgcacgccattctgcggcggcaggaagatttttacccattcctgaaggacaaccgggaaaagatcgagaagatcctgaccttccgcatcccctactacgtgggccctctggccaggggaaacagcagattcgcctggatgaccagaaagagcgaggaaaccatcaccccctggaacttcgaggaagtggtggacaagggcgcttccgcccagagcttcatcgagcggatgaccaacttcgataagaacctgcccaacgagaaggtgctgcccaagcacagcctgctgtacgagtacttcaccgtgtataacgagctgaccaaagtgaaatacgtgaccgagggaatgagaaagcccgccttcctgagcggcgagcagaaaaaggccatcgtggacctgctgttcaagaccaaccggaaagtgaccgtgaagcagctgaaagaggactacttcaagaaaatcgagtgcttcgactccgtggaaatctccggcgtggaagatcggttcaacgcctccctgggcacataccacgatctgctgaaaattatcaaggacaaggacttcctggacaatgaggaaaacgaggacattctggaagatatcgtgctgaccctgacactgtttgaggacagagagatgatcgaggaacggctgaaaacctatgcccacctgttcgacgacaaagtgatgaagcagctgaagcggcggagatacaccggctggggcaggctgagccggaagctgatcaacggcatccgggacaagcagtccggcaagacaatcctggatttcctgaagtccgacggcttcgccaacagaaacttcatgcagctgatccacgacgacagcctgacctttaaagaggacatccagaaagcccaggtgtccggccagggcgatagcctgcacgagcacattgccaatctggccggcagccccgccattaagaagggcatcctgcagacagtgaaggtggtggacgagctcgtgaaagtgatgggccggcacaagcccgagaacatcgtgatcgaaatggccagagagaaccagaccacccagaagggacagaagaacagccgcgagagaatgaagcggatcgaagagggcatcaaagagctgggcagccagatcctgaaagaacaccccgtggaaaacacccagctgcagaacgagaagctgtacctgtactacctgcagaatgggcgggatatgtacgtggaccaggaactggacatcaaccggctgtccgactacgatgtggaccatatcgtgcctcagagctttctgaaggacgactccatcgacaacaaggtgctgaccagaagcgacaagaaccggggcaagagcgacaacgtgccctccgaagaggtcgtgaagaagatgaagaactactggcggcagctgctgaacgccaagctgattacccagagaaagttcgacaatctgaccaaggccgagagaggcggcctgagcgaactggataaggccggcttcatcaagagacagctggtggaaacccggcagatcacaaagcacgtggcacagatcctggactcccggatgaacactaagtacgacgagaatgacaagctgatccgggaagtgaaagtgatcaccctgaagtccaagctggtgtccgatttccggaaggatttccagttttacaaagtgcgcgagatcaacaactaccaccacgcccacgacgcctacctgaacgccgtcgtgggaaccgccctgatcaaaaagtaccctaagctggaaagcgagttcgtgtacggcgactacaaggtgtacgacgtgcggaagatgatcgccaagagcgagcaggaaatcggcaaggctaccgccaagtacttcttctacagcaacatcatgaactttttcaagaccgagattaccctggccaacggcgagatccggaagcggcctctgatcgagacaaacggcgaaaccggggagatcgtgtgggataagggccgggattttgccaccgtgcggaaagtgctgagcatgccccaagtgaatatcgtgaaaaagaccgaggtgcagacaggcggcttcagcaaagagtctatcctgcccaagaggaacagcgataagctgatcgccagaaagaaggactgggaccctaagaagtacggcggcttcgacagccccaccgtggcctattctgtgctggtggtggccaaagtggaaaagggcaagtccaagaaactgaagagtgtgaaagagctgctggggatcaccatcatggaaagaagcagcttcgagaagaatcccatcgactttctggaagccaagggctacaaagaagtgaaaaaggacctgatcatcaagctgcctaagtactccctgttcgagctggaaaacggccggaagagaatgctggcctctgccggcgaactgcagaagggaaacgaactggccctgccctccaaatatgtgaacttcctgtacctggccagccactatgagaagctgaagggctcccccgaggataatgagcagaaacagctgtttgtggaacagcacaagcactacctggacgagatcatcgagcagatcagcgagttctccaagagagtgatcctggccgacgctaatctggacaaagtgctgtccgcctacaacaagcaccgggataagcccatcagagagcaggccgagaatatcatccacctgtttaccctgaccaatctgggagcccctgccgccttcaagtactttgacaccaccatcgaccggaagaggtacaccagcaccaaagaggtgctggacgccaccctgatccaccagagcatcaccggcctgtacgagacacggatcgacctgtctcagctgggaggcgacgatccaaaaaagaagagaaaggtaggcggctctggcggcggctccggaggctctgagatcgccgccctggaggccaagatcgccgccctgaaggccaagaacgccgccctgaaggccgagatcgccgccctggaggcctaa

SEQ ID NO: 4 - DNA, 4293 bp, Artificial Sequence
  Cas9-N6
atggccccaaagaagaagcggaaggtcggtatccacggagtcccagcagccgacaagaagtacagcatcggcctggacatcggcaccaactctgtgggctgggccgtgatcaccgacgagtacaaggtgcccagcaagaaattcaaggtgctgggcaacaccgaccggcacagcatcaagaagaacctgatcggagccctgctgttcgacagcggcgaaacagccgaggccacccggctgaagagaaccgccagaagaagatacaccagacggaagaaccggatctgctatctgcaagagatcttcagcaacgagatggccaaggtggacgacagcttcttccacagactggaagagtccttcctggtggaagaggataagaagcacgagcggcaccccatcttcggcaacatcgtggacgaggtggcctaccacgagaagtaccccaccatctaccacctgagaaagaaactggtggacagcaccgacaaggccgacctgcggctgatctatctggccctggcccacatgatcaagttccggggccacttcctgatcgagggcgacctgaaccccgacaacagcgacgtggacaagctgttcatccagctggtgcagacctacaaccagctgttcgaggaaaaccccatcaacgccagcggcgtggacgccaaggccatcctgtctgccagactgagcaagagcagacggctggaaaatctgatcgcccagctgcccggcgagaagaagaatggcctgttcggaaacctgattgccctgagcctgggcctgacccccaacttcaagagcaacttcgacctggccgaggatgccaaactgcagctgagcaaggacacctacgacgacgacctggacaacctgctggcccagatcggcgaccagtacgccgacctgtttctggccgccaagaacctgtccgacgccatcctgctgagcgacatcctgagagtgaacaccgagatcaccaaggcccccctgagcgcctctatgatcaagagatacgacgagcaccaccaggacctgaccctgctgaaagctctcgtgcggcagcagctgcctgagaagtacaaagagattttcttcgaccagagcaagaacggctacgccggctacattgacggcggagccagccaggaagagttctacaagttcatcaagcccatcctggaaaagatggacggcaccgaggaactgctcgtgaagctgaacagagaggacctgctgcggaagcagcggaccttcgacaacggcagcatcccccaccagatccacctgggagagctgcacgccattctgcggcggcaggaagatttttacccattcctgaaggacaaccgggaaaagatcgagaagatcctgaccttccgcatcccctactacgtgggccctctggccaggggaaacagcagattcgcctggatgaccagaaagagcgaggaaaccatcaccccctggaacttcgaggaagtggtggacaagggcgcttccgcccagagcttcatcgagcggatgaccaacttcgataagaacctgcccaacgagaaggtgctgcccaagcacagcctgctgtacgagtacttcaccgtgtataacgagctgaccaaagtgaaatacgtgaccgagggaatgagaaagcccgccttcctgagcggcgagcagaaaaaggccatcgtggacctgctgttcaagaccaaccggaaagtgaccgtgaagcagctgaaagaggactacttcaagaaaatcgagtgcttcgactccgtggaaatctccggcgtggaagatcggttcaacgcctccctgggcacataccacgatctgctgaaaattatcaaggacaaggacttcctggacaatgaggaaaacgaggacattctggaagatatcgtgctgaccctgacactgtttgaggacagagagatgatcgaggaacggctgaaaacctatgcccacctgttcgacgacaaagtgatgaagcagctgaagcggcggagatacaccggctggggcaggctgagccggaagctgatcaacggcatccgggacaagcagtccggcaagacaatcctggatttcctgaagtccgacggcttcgccaacagaaacttcatgcagctgatccacgacgacagcctgacctttaaagaggacatccagaaagcccaggtgtccggccagggcgatagcctgcacgagcacattgccaatctggccggcagccccgccattaagaagggcatcctgcagacagtgaaggtggtggacgagctcgtgaaagtgatgggccggcacaagcccgagaacatcgtgatcgaaatggccagagagaaccagaccacccagaagggacagaagaacagccgcgagagaatgaagcggatcgaagagggcatcaaagagctgggcagccagatcctgaaagaacaccccgtggaaaacacccagctgcagaacgagaagctgtacctgtactacctgcagaatgggcgggatatgtacgtggaccaggaactggacatcaaccggctgtccgactacgatgtggaccatatcgtgcctcagagctttctgaaggacgactccatcgacaacaaggtgctgaccagaagcgacaagaaccggggcaagagcgacaacgtgccctccgaagaggtcgtgaagaagatgaagaactactggcggcagctgctgaacgccaagctgattacccagagaaagttcgacaatctgaccaaggccgagagaggcggcctgagcgaactggataaggccggcttcatcaagagacagctggtggaaacccggcagatcacaaagcacgtggcacagatcctggactcccggatgaacactaagtacgacgagaatgacaagctgatccgggaagtgaaagtgatcaccctgaagtccaagctggtgtccgatttccggaaggatttccagttttacaaagtgcgcgagatcaacaactaccaccacgcccacgacgcctacctgaacgccgtcgtgggaaccgccctgatcaaaaagtaccctaagctggaaagcgagttcgtgtacggcgactacaaggtgtacgacgtgcggaagatgatcgccaagagcgagcaggaaatcggcaaggctaccgccaagtacttcttctacagcaacatcatgaactttttcaagaccgagattaccctggccaacggcgagatccggaagcggcctctgatcgagacaaacggcgaaaccggggagatcgtgtgggataagggccgggattttgccaccgtgcggaaagtgctgagcatgccccaagtgaatatcgtgaaaaagaccgaggtgcagacaggcggcttcagcaaagagtctatcctgcccaagaggaacagcgataagctgatcgccagaaagaaggactgggaccctaagaagtacggcggcttcgacagccccaccgtggcctattctgtgctggtggtggccaaagtggaaaagggcaagtccaagaaactgaagagtgtgaaagagctgctggggatcaccatcatggaaagaagcagcttcgagaagaatcccatcgactttctggaagccaagggctacaaagaagtgaaaaaggacctgatcatcaagctgcctaagtactccctgttcgagctggaaaacggccggaagagaatgctggcctctgccggcgaactgcagaagggaaacgaactggccctgccctccaaatatgtgaacttcctgtacctggccagccactatgagaagctgaagggctcccccgaggataatgagcagaaacagctgtttgtggaacagcacaagcactacctggacgagatcatcgagcagatcagcgagttctccaagagagtgatcctggccgacgctaatctggacaaagtgctgtccgcctacaacaagcaccgggataagcccatcagagagcaggccgagaatatcatccacctgtttaccctgaccaatctgggagcccctgccgccttcaagtactttgacaccaccatcgaccggaagaggtacaccagcaccaaagaggtgctggacgccaccctgatccaccagagcatcaccggcctgtacgagacacggatcgacctgtctcagctgggaggcgacgatccaaaaaagaagagaaaggtaggcggctctggcggcggctccggaggctctaagatcgccgccctgaaggccgagatcgccgccctggaggccgagaacgccgccctggaggccaagatcgccgccctgaaggcctaa

SEQ ID NO: 5 - DNA, 4305 bp, Artificial Sequence
  Cas9-P3S
atggccccaaagaagaagcggaaggtcggtatccacggagtcccagcagccgacaagaagtacagcatcggcctggacatcggcaccaactctgtgggctgggccgtgatcaccgacgagtacaaggtgcccagcaagaaattcaaggtgctgggcaacaccgaccggcacagcatcaagaagaacctgatcggagccctgctgttcgacagcggcgaaacagccgaggccacccggctgaagagaaccgccagaagaagatacaccagacggaagaaccggatctgctatctgcaagagatcttcagcaacgagatggccaaggtggacgacagcttcttccacagactggaagagtccttcctggtggaagaggataagaagcacgagcggcaccccatcttcggcaacatcgtggacgaggtggcctaccacgagaagtaccccaccatctaccacctgagaaagaaactggtggacagcaccgacaaggccgacctgcggctgatctatctggccctggcccacatgatcaagttccggggccacttcctgatcgagggcgacctgaaccccgacaacagcgacgtggacaagctgttcatccagctggtgcagacctacaaccagctgttcgaggaaaaccccatcaacgccagcggcgtggacgccaaggccatcctgtctgccagactgagcaagagcagacggctggaaaatctgatcgcccagctgcccggcgagaagaagaatggcctgttcggaaacctgattgccctgagcctgggcctgacccccaacttcaagagcaacttcgacctggccgaggatgccaaactgcagctgagcaaggacacctacgacgacgacctggacaacctgctggcccagatcggcgaccagtacgccgacctgtttctggccgccaagaacctgtccgacgccatcctgctgagcgacatcctgagagtgaacaccgagatcaccaaggcccccctgagcgcctctatgatcaagagatacgacgagcaccaccaggacctgaccctgctgaaagctctcgtgcggcagcagctgcctgagaagtacaaagagattttcttcgaccagagcaagaacggctacgccggctacattgacggcggagccagccaggaagagttctacaagttcatcaagcccatcctggaaaagatggacggcaccgaggaactgctcgtgaagctgaacagagaggacctgctgcggaagcagcggaccttcgacaacggcagcatcccccaccagatccacctgggagagctgcacgccattctgcggcggcaggaagatttttacccattcctgaaggacaaccgggaaaagatcgagaagatcctgaccttccgcatcccctactacgtgggccctctggccaggggaaacagcagattcgcctggatgaccagaaagagcgaggaaaccatcaccccctggaacttcgaggaagtggtggacaagggcgcttccgcccagagcttcatcgagcggatgaccaacttcgataagaacctgcccaacgagaaggtgctgcccaagcacagcctgctgtacgagtacttcaccgtgtataacgagctgaccaaagtgaaatacgtgaccgagggaatgagaaagcccgccttcctgagcggcgagcagaaaaaggccatcgtggacctgctgttcaagaccaaccggaaagtgaccgtgaagcagctgaaagaggactacttcaagaaaatcgagtgcttcgactccgtggaaatctccggcgtggaagatcggttcaacgcctccctgggcacataccacgatctgctgaaaattatcaaggacaaggacttcctggacaatgaggaaaacgaggacattctggaagatatcgtgctgaccctgacactgtttgaggacagagagatgatcgaggaacggctgaaaacctatgcccacctgttcgacgacaaagtgatgaagcagctgaagcggcggagatacaccggctggggcaggctgagccggaagctgatcaacggcatccgggacaagcagtccggcaagacaatcctggatttcctgaagtccgacggcttcgccaacagaaacttcatgcagctgatccacgacgacagcctgacctttaaagaggacatccagaaagcccaggtgtccggccagggcgatagcctgcacgagcacattgccaatctggccggcagccccgccattaagaagggcatcctgcagacagtgaaggtggtggacgagctcgtgaaagtgatgggccggcacaagcccgagaacatcgtgatcgaaatggccagagagaaccagaccacccagaagggacagaagaacagccgcgagagaatgaagcggatcgaagagggcatcaaagagctgggcagccagatcctgaaagaacaccccgtggaaaacacccagctgcagaacgagaagctgtacctgtactacctgcagaatgggcgggatatgtacgtggaccaggaactggacatcaaccggctgtccgactacgatgtggaccatatcgtgcctcagagctttctgaaggacgactccatcgacaacaaggtgctgaccagaagcgacaagaaccggggcaagagcgacaacgtgccctccgaagaggtcgtgaagaagatgaagaactactggcggcagctgctgaacgccaagctgattacccagagaaagttcgacaatctgaccaaggccgagagaggcggcctgagcgaactggataaggccggcttcatcaagagacagctggtggaaacccggcagatcacaaagcacgtggcacagatcctggactcccggatgaacactaagtacgacgagaatgacaagctgatccgggaagtgaaagtgatcaccctgaagtccaagctggtgtccgatttccggaaggatttccagttttacaaagtgcgcgagatcaacaactaccaccacgcccacgacgcctacctgaacgccgtcgtgggaaccgccctgatcaaaaagtaccctaagctggaaagcgagttcgtgtacggcgactacaaggtgtacgacgtgcggaagatgatcgccaagagcgagcaggaaatcggcaaggctaccgccaagtacttcttctacagcaacatcatgaactttttcaagaccgagattaccctggccaacggcgagatccggaagcggcctctgatcgagacaaacggcgaaaccggggagatcgtgtgggataagggccgggattttgccaccgtgcggaaagtgctgagcatgccccaagtgaatatcgtgaaaaagaccgaggtgcagacaggcggcttcagcaaagagtctatcctgcccaagaggaacagcgataagctgatcgccagaaagaaggactgggaccctaagaagtacggcggcttcgacagccccaccgtggcctattctgtgctggtggtggccaaagtggaaaagggcaagtccaagaaactgaagagtgtgaaagagctgctggggatcaccatcatggaaagaagcagcttcgagaagaatcccatcgactttctggaagccaagggctacaaagaagtgaaaaaggacctgatcatcaagctgcctaagtactccctgttcgagctggaaaacggccggaagagaatgctggcctctgccggcgaactgcagaagggaaacgaactggccctgccctccaaatatgtgaacttcctgtacctggccagccactatgagaagctgaagggctcccccgaggataatgagcagaaacagctgtttgtggaacagcacaagcactacctggacgagatcatcgagcagatcagcgagttctccaagagagtgatcctggccgacgctaatctggacaaagtgctgtccgcctacaacaagcaccgggataagcccatcagagagcaggccgagaatatcatccacctgtttaccctgaccaatctgggagcccctgccgccttcaagtactttgacaccaccatcgaccggaagaggtacaccagcaccaaagaggtgctggacgccaccctgatccaccagagcatcaccggcctgtacgagacacggatcgacctgtctcagctgggaggcgacgatccaaaaaagaagagaaaggtaggcggctctggcggcggctccggaggctctagccccgaggacgagatccagcagctggaggaggagatcagccagctggagcagaagaacagccagctgaaggagaagaaccagcagctgaagtactaa

SEQ ID NO: 6 - DNA, 4305 bp, Artificial Sequence
  Cas9-P4S
atggccccaaagaagaagcggaaggtcggtatccacggagtcccagcagccgacaagaagtacagcatcggcctggacatcggcaccaactctgtgggctgggccgtgatcaccgacgagtacaaggtgcccagcaagaaattcaaggtgctgggcaacaccgaccggcacagcatcaagaagaacctgatcggagccctgctgttcgacagcggcgaaacagccgaggccacccggctgaagagaaccgccagaagaagatacaccagacggaagaaccggatctgctatctgcaagagatcttcagcaacgagatggccaaggtggacgacagcttcttccacagactggaagagtccttcctggtggaagaggataagaagcacgagcggcaccccatcttcggcaacatcgtggacgaggtggcctaccacgagaagtaccccaccatctaccacctgagaaagaaactggtggacagcaccgacaaggccgacctgcggctgatctatctggccctggcccacatgatcaagttccggggccacttcctgatcgagggcgacctgaaccccgacaacagcgacgtggacaagctgttcatccagctggtgcagacctacaaccagctgttcgaggaaaaccccatcaacgccagcggcgtggacgccaaggccatcctgtctgccagactgagcaagagcagacggctggaaaatctgatcgcccagctgcccggcgagaagaagaatggcctgttcggaaacctgattgccctgagcctgggcctgacccccaacttcaagagcaacttcgacctggccgaggatgccaaactgcagctgagcaaggacacctacgacgacgacctggacaacctgctggcccagatcggcgaccagtacgccgacctgtttctggccgccaagaacctgtccgacgccatcctgctgagcgacatcctgagagtgaacaccgagatcaccaaggcccccctgagcgcctctatgatcaagagatacgacgagcaccaccaggacctgaccctgctgaaagctctcgtgcggcagcagctgcctgagaagtacaaagagattttcttcgaccagagcaagaacggctacgccggctacattgacggcggagccagccaggaagagttctacaagttcatcaagcccatcctggaaaagatggacggcaccgaggaactgctcgtgaagctgaacagagaggacctgctgcggaagcagcggaccttcgacaacggcagcatcccccaccagatccacctgggagagctgcacgccattctgcggcggcaggaagatttttacccattcctgaaggacaaccgggaaaagatcgagaagatcctgaccttccgcatcccctactacgtgggccctctggccaggggaaacagcagattcgcctggatgaccagaaagagcgaggaaaccatcaccccctggaacttcgaggaagtggtggacaagggcgcttccgcccagagcttcatcgagcggatgaccaacttcgataagaacctgcccaacgagaaggtgctgcccaagcacagcctgctgtacgagtacttcaccgtgtataacgagctgaccaaagtgaaatacgtgaccgagggaatgagaaagcccgccttcctgagcggcgagcagaaaaaggccatcgtggacctgctgttcaagaccaaccggaaagtgaccgtgaagcagctgaaagaggactacttcaagaaaatcgagtgcttcgactccgtggaaatctccggcgtggaagatcggttcaacgcctccctgggcacataccacgatctgctgaaaattatcaaggacaaggacttcctggacaatgaggaaaacgaggacattctggaagatatcgtgctgaccctgacactgtttgaggacagagagatgatcgaggaacggctgaaaacctatgcccacctgttcgacgacaaagtgatgaagcagctgaagcggcggagatacaccggctggggcaggctgagccggaagctgatcaacggcatccgggacaagcagtccggcaagacaatcctggatttcctgaagtccgacggcttcgccaacagaaacttcatgcagctgatccacgacgacagcctgacctttaaagaggacatccagaaagcccaggtgtccggccagggcgatagcctgcacgagcacattgccaatctggccggcagccccgccattaagaagggcatcctgcagacagtgaaggtggtggacgagctcgtgaaagtgatgggccggcacaagcccgagaacatcgtgatcgaaatggccagagagaaccagaccacccagaagggacagaagaacagccgcgagagaatgaagcggatcgaagagggcatcaaagagctgggcagccagatcctgaaagaacaccccgtggaaaacacccagctgcagaacgagaagctgtacctgtactacctgcagaatgggcgggatatgtacgtggaccaggaactggacatcaaccggctgtccgactacgatgtggaccatatcgtgcctcagagctttctgaaggacgactccatcgacaacaaggtgctgaccagaagcgacaagaaccggggcaagagcgacaacgtgccctccgaagaggtcgtgaagaagatgaagaactactggcggcagctgctgaacgccaagctgattacccagagaaagttcgacaatctgaccaaggccgagagaggcggcctgagcgaactggataaggccggcttcatcaagagacagctggtggaaacccggcagatcacaaagcacgtggcacagatcctggactcccggatgaacactaagtacgacgagaatgacaagctgatccgggaagtgaaagtgatcaccctgaagtccaagctggtgtccgatttccggaaggatttccagttttacaaagtgcgcgagatcaacaactaccaccacgcccacgacgcctacctgaacgccgtcgtgggaaccgccctgatcaaaaagtaccctaagctggaaagcgagttcgtgtacggcgactacaaggtgtacgacgtgcggaagatgatcgccaagagcgagcaggaaatcggcaaggctaccgccaagtacttcttctacagcaacatcatgaactttttcaagaccgagattaccctggccaacggcgagatccggaagcggcctctgatcgagacaaacggcgaaaccggggagatcgtgtgggataagggccgggattttgccaccgtgcggaaagtgctgagcatgccccaagtgaatatcgtgaaaaagaccgaggtgcagacaggcggcttcagcaaagagtctatcctgcccaagaggaacagcgataagctgatcgccagaaagaaggactgggaccctaagaagtacggcggcttcgacagccccaccgtggcctattctgtgctggtggtggccaaagtggaaaagggcaagtccaagaaactgaagagtgtgaaagagctgctggggatcaccatcatggaaagaagcagcttcgagaagaatcccatcgactttctggaagccaagggctacaaagaagtgaaaaaggacctgatcatcaagctgcctaagtactccctgttcgagctggaaaacggccggaagagaatgctggcctctgccggcgaactgcagaagggaaacgaactggccctgccctccaaatatgtgaacttcctgtacctggccagccactatgagaagctgaagggctcccccgaggataatgagcagaaacagctgtttgtggaacagcacaagcactacctggacgagatcatcgagcagatcagcgagttctccaagagagtgatcctggccgacgctaatctggacaaagtgctgtccgcctacaacaagcaccgggataagcccatcagagagcaggccgagaatatcatccacctgtttaccctgaccaatctgggagcccctgccgccttcaagtactttgacaccaccatcgaccggaagaggtacaccagcaccaaagaggtgctggacgccaccctgatccaccagagcatcaccggcctgtacgagacacggatcgacctgtctcagctgggaggcgacgatccaaaaaagaagagaaaggtaggcggctctggcggcggctccggaggctctagccccgaggacaagatcagccagctgaagcagaagatccagcagctgaagcaggagaaccagcagctggaggaggagaacagccagctggagtactaa

SEQ ID NO: 7 - DNA, 4305 bp, Artificial Sequence
  Cas9-AP4
atggccccaaagaagaagcggaaggtcggtatccacggagtcccagcagccgacaagaagtacagcatcggcctggacatcggcaccaactctgtgggctgggccgtgatcaccgacgagtacaaggtgcccagcaagaaattcaaggtgctgggcaacaccgaccggcacagcatcaagaagaacctgatcggagccctgctgttcgacagcggcgaaacagccgaggccacccggctgaagagaaccgccagaagaagatacaccagacggaagaaccggatctgctatctgcaagagatcttcagcaacgagatggccaaggtggacgacagcttcttccacagactggaagagtccttcctggtggaagaggataagaagcacgagcggcaccccatcttcggcaacatcgtggacgaggtggcctaccacgagaagtaccccaccatctaccacctgagaaagaaactggtggacagcaccgacaaggccgacctgcggctgatctatctggccctggcccacatgatcaagttccggggccacttcctgatcgagggcgacctgaaccccgacaacagcgacgtggacaagctgttcatccagctggtgcagacctacaaccagctgttcgaggaaaaccccatcaacgccagcggcgtggacgccaaggccatcctgtctgccagactgagcaagagcagacggctggaaaatctgatcgcccagctgcccggcgagaagaagaatggcctgttcggaaacctgattgccctgagcctgggcctgacccccaacttcaagagcaacttcgacctggccgaggatgccaaactgcagctgagcaaggacacctacgacgacgacctggacaacctgctggcccagatcggcgaccagtacgccgacctgtttctggccgccaagaacctgtccgacgccatcctgctgagcgacatcctgagagtgaacaccgagatcaccaaggcccccctgagcgcctctatgatcaagagatacgacgagcaccaccaggacctgaccctgctgaaagctctcgtgcggcagcagctgcctgagaagtacaaagagattttcttcgaccagagcaagaacggctacgccggctacattgacggcggagccagccaggaagagttctacaagttcatcaagcccatcctggaaaagatggacggcaccgaggaactgctcgtgaagctgaacagagaggacctgctgcggaagcagcggaccttcgacaacggcagcatcccccaccagatccacctgggagagctgcacgccattctgcggcggcaggaagatttttacccattcctgaaggacaaccgggaaaagatcgagaagatcctgaccttccgcatcccctactacgtgggccctctggccaggggaaacagcagattcgcctggatgaccagaaagagcgaggaaaccatcaccccctggaacttcgaggaagtggtggacaagggcgcttccgcccagagcttcatcgagcggatgaccaacttcgataagaacctgcccaacgagaaggtgctgcccaagcacagcctgctgtacgagtacttcaccgtgtataacgagctgaccaaagtgaaatacgtgaccgagggaatgagaaagcccgccttcctgagcggcgagcagaaaaaggccatcgtggacctgctgttcaagaccaaccggaaagtgaccgtgaagcagctgaaagaggactacttcaagaaaatcgagtgcttcgactccgtggaaatctccggcgtggaagatcggttcaacgcctccctgggcacataccacgatctgctgaaaattatcaaggacaaggacttcctggacaatgaggaaaacgaggacattctggaagatatcgtgctgaccctgacactgtttgaggacagagagatgatcgaggaacggctgaaaacctatgcccacctgttcgacgacaaagtgatgaagcagctgaagcggcggagatacaccggctggggcaggctgagccggaagctgatcaacggcatccgggacaagcagtccggcaagacaatcctggatttcctgaagtccgacggcttcgccaacagaaacttcatgcagctgatccacgacgacagcctgacctttaaagaggacatccagaaagcccaggtgtccggccagggcgatagcctgcacgagcacattgccaatctggccggcagccccgccattaagaagggcatcctgcagacagtgaaggtggtggacgagctcgtgaaagtgatgggccggcacaagcccgagaacatcgtgatcgaaatggccagagagaaccagaccacccagaagggacagaagaacagccgcgagagaatgaagcggatcgaagagggcatcaaagagctgggcagccagatcctgaaagaacaccccgtggaaaacacccagctgcagaacgagaagctgtacctgtactacctgcagaatgggcgggatatgtacgtggaccaggaactggacatcaaccggctgtccgactacgatgtggaccatatcgtgcctcagagctttctgaaggacgactccatcgacaacaaggtgctgaccagaagcgacaagaaccggggcaagagcgacaacgtgccctccgaagaggtcgtgaagaagatgaagaactactggcggcagctgctgaacgccaagctgattacccagagaaagttcgacaatctgaccaaggccgagagaggcggcctgagcgaactggataaggccggcttcatcaagagacagctggtggaaacccggcagatcacaaagcacgtggcacagatcctggactcccggatgaacactaagtacgacgagaatgacaagctgatccgggaagtgaaagtgatcaccctgaagtccaagctggtgtccgatttccggaaggatttccagttttacaaagtgcgcgagatcaacaactaccaccacgcccacgacgcctacctgaacgccgtcgtgggaaccgccctgatcaaaaagtaccctaagctggaaagcgagttcgtgtacggcgactacaaggtgtacgacgtgcggaagatgatcgccaagagcgagcaggaaatcggcaaggctaccgccaagtacttcttctacagcaacatcatgaactttttcaagaccgagattaccctggccaacggcgagatccggaagcggcctctgatcgagacaaacggcgaaaccggggagatcgtgtgggataagggccgggattttgccaccgtgcggaaagtgctgagcatgccccaagtgaatatcgtgaaaaagaccgaggtgcagacaggcggcttcagcaaagagtctatcctgcccaagaggaacagcgataagctgatcgccagaaagaaggactgggaccctaagaagtacggcggcttcgacagccccaccgtggcctattctgtgctggtggtggccaaagtggaaaagggcaagtccaagaaactgaagagtgtgaaagagctgctggggatcaccatcatggaaagaagcagcttcgagaagaatcccatcgactttctggaagccaagggctacaaagaagtgaaaaaggacctgatcatcaagctgcctaagtactccctgttcgagctggaaaacggccggaagagaatgctggcctctgccggcgaactgcagaagggaaacgaactggccctgccctccaaatatgtgaacttcctgtacctggccagccactatgagaagctgaagggctcccccgaggataatgagcagaaacagctgtttgtggaacagcacaagcactacctggacgagatcatcgagcagatcagcgagttctccaagagagtgatcctggccgacgctaatctggacaaagtgctgtccgcctacaacaagcaccgggataagcccatcagagagcaggccgagaatatcatccacctgtttaccctgaccaatctgggagcccctgccgccttcaagtactttgacaccaccatcgaccggaagaggtacaccagcaccaaagaggtgctggacgccaccctgatccaccagagcatcaccggcctgtacgagacacggatcgacctgtctcagctgggaggcgacgatccaaaaaagaagagaaaggtaggcggctctggcggcggctccggaggctctagccccgaggacgagctggccgccaacgaggaggagctgcagcagaacgagcagaagctggcccagatcaagcagaagctgcaggccatcaagtactaa

SEQ ID NO: 8 - DNA, 957 bp, Artificial Sequence
  P4-EXOIII
agcccggaagataaaattgctcagctgaaacaaaaaatccaagcgctgaaacaggaaaaccagcagctggaagaggaaaacgccgcactggaatatggtggcggctctggcggcggctccggaggctctgatccaaaaaagaagagaaaggtaaaatttgtctcttttaatatcaacggcctgcgcgccagacctcaccagcttgaagccatcgtcgaaaagcaccaaccggatgtgattggcctgcaggagacaaaagttcatgacgatatgtttccgctcgaagaggtggcgaagctcggctacaacgtgttttatcacgggcagaaaggccattatggcgtggcgctgctgaccaaagagacgccgattgccgtgcgtcgcggctttcccggtgacgacgaagaggcgcagcggcggattattatggcggaaatcccctcactgctgggtaatgtcaccgtgatcaacggttacttcccgcagggtgaaagccgcgaccatccgataaaattcccggcaaaagcgcagttttatcagaatctgcaaaactacctggaaaccgaactcaaacgtgataatccggtactgattatgggcgatatgaatatcagccctacagatctggacatcggcattggcgaagaaaaccgtaagcgctggctgcgtaccggtaaatgctctttcctgccggaagagcgcgaatggatggacaggctgatgagctgggggttggtcgataccttccgccatgcgaatccgcaaacagcagatcgtttctcatggtttgattaccgctcaaaaggttttgacgataaccgtggtctgcgcatcgacctgctgctcgccagccaaccgctggcagaatgttgcgtagaaaccggcatcgactatgaaatccgcagcatggaaaaaccgtccgatcacgcccccgtctgggcgaccttccgccgctaa

SEQ ID NO: 9 - DNA, 957 bp, Artificial Sequence
  P3-EXOIII
tccccggaagatgagatccagcaactggaagaagaaatcgctcagctggaacagaaaaacgcagcgctgaaagagaaaaaccaggcgctgaaatacggtggcggctctggcggcggctccggaggctctgatccaaaaaagaagagaaaggtaaaatttgtctcttttaatatcaacggcctgcgcgccagacctcaccagcttgaagccatcgtcgaaaagcaccaaccggatgtgattggcctgcaggagacaaaagttcatgacgatatgtttccgctcgaagaggtggcgaagctcggctacaacgtgttttatcacgggcagaaaggccattatggcgtggcgctgctgaccaaagagacgccgattgccgtgcgtcgcggctttcccggtgacgacgaagaggcgcagcggcggattattatggcggaaatcccctcactgctgggtaatgtcaccgtgatcaacggttacttcccgcagggtgaaagccgcgaccatccgataaaattcccggcaaaagcgcagttttatcagaatctgcaaaactacctggaaaccgaactcaaacgtgataatccggtactgattatgggcgatatgaatatcagccctacagatctggacatcggcattggcgaagaaaaccgtaagcgctggctgcgtaccggtaaatgctctttcctgccggaagagcgcgaatggatggacaggctgatgagctgggggttggtcgataccttccgccatgcgaatccgcaaacagcagatcgtttctcatggtttgattaccgctcaaaaggttttgacgataaccgtggtctgcgcatcgacctgctgctcgccagccaaccgctggcagaatgttgcgtagaaaccggcatcgactatgaaatccgcagcatggaaaaaccgtccgatcacgcccccgtctgggcgaccttccgccgctaa

SEQ ID NO: 10 - DNA, 939 bp, Artificial Sequence
  N5-EXOIII
gagatcgccgccctggaggccaagatcgccgccctgaaggccaagaacgccgccctgaaggccgagatcgccgccctggaggccggcggctctggcggcggctccggaggctctgatccaaaaaagaagagaaaggtaaaatttgtctcttttaatatcaacggcctgcgcgccagacctcaccagcttgaagccatcgtcgaaaagcaccaaccggatgtgattggcctgcaggagacaaaagttcatgacgatatgtttccgctcgaagaggtggcgaagctcggctacaacgtgttttatcacgggcagaaaggccattatggcgtggcgctgctgaccaaagagacgccgattgccgtgcgtcgcggctttcccggtgacgacgaagaggcgcagcggcggattattatggcggaaatcccctcactgctgggtaatgtcaccgtgatcaacggttacttcccgcagggtgaaagccgcgaccatccgataaaattcccggcaaaagcgcagttttatcagaatctgcaaaactacctggaaaccgaactcaaacgtgataatccggtactgattatgggcgatatgaatatcagccctacagatctggacatcggcattggcgaagaaaaccgtaagcgctggctgcgtaccggtaaatgctctttcctgccggaagagcgcgaatggatggacaggctgatgagctgggggttggtcgataccttccgccatgcgaatccgcaaacagcagatcgtttctcatggtttgattaccgctcaaaaggttttgacgataaccgtggtctgcgcatcgacctgctgctcgccagccaaccgctggcagaatgttgcgtagaaaccggcatcgactatgaaatccgcagcatggaaaaaccgtccgatcacgcccccgtctgggcgaccttccgccgc

SEQ ID NO: 11 - DNA, 939 bp, Artificial Sequence
  N6-EXOIII
aagatcgccgccctgaaggccgagatcgccgccctggaggccgagaacgccgccctggaggccaagatcgccgccctgaaggccggcggctctggcggcggctccggaggctctgatccaaaaaagaagagaaaggtaaaatttgtctcttttaatatcaacggcctgcgcgccagacctcaccagcttgaagccatcgtcgaaaagcaccaaccggatgtgattggcctgcaggagacaaaagttcatgacgatatgtttccgctcgaagaggtggcgaagctcggctacaacgtgttttatcacgggcagaaaggccattatggcgtggcgctgctgaccaaagagacgccgattgccgtgcgtcgcggctttcccggtgacgacgaagaggcgcagcggcggattattatggcggaaatcccctcactgctgggtaatgtcaccgtgatcaacggttacttcccgcagggtgaaagccgcgaccatccgataaaattcccggcaaaagcgcagttttatcagaatctgcaaaactacctggaaaccgaactcaaacgtgataatccggtactgattatgggcgatatgaatatcagccctacagatctggacatcggcattggcgaagaaaaccgtaagcgctggctgcgtaccggtaaatgctctttcctgccggaagagcgcgaatggatggacaggctgatgagctgggggttggtcgataccttccgccatgcgaatccgcaaacagcagatcgtttctcatggtttgattaccgctcaaaaggttttgacgataaccgtggtctgcgcatcgacctgctgctcgccagccaaccgctggcagaatgttgcgtagaaaccggcatcgactatgaaatccgcagcatggaaaaaccgtccgatcacgcccccgtctgggcgaccttccgccgc

SEQ ID NO: 12 - DNA, 951 bp, Artificial Sequence
  P3S-EXOIII
agccccgaggacgagatccagcagctggaggaggagatcagccagctggagcagaagaacagccagctgaaggagaagaaccagcagctgaagtacggcggctctggcggcggctccggaggctctgatccaaaaaagaagagaaaggtaaaatttgtctcttttaatatcaacggcctgcgcgccagacctcaccagcttgaagccatcgtcgaaaagcaccaaccggatgtgattggcctgcaggagacaaaagttcatgacgatatgtttccgctcgaagaggtggcgaagctcggctacaacgtgttttatcacgggcagaaaggccattatggcgtggcgctgctgaccaaagagacgccgattgccgtgcgtcgcggctttcccggtgacgacgaagaggcgcagcggcggattattatggcggaaatcccctcactgctgggtaatgtcaccgtgatcaacggttacttcccgcagggtgaaagccgcgaccatccgataaaattcccggcaaaagcgcagttttatcagaatctgcaaaactacctggaaaccgaactcaaacgtgataatccggtactgattatgggcgatatgaatatcagccctacagatctggacatcggcattggcgaagaaaaccgtaagcgctggctgcgtaccggtaaatgctctttcctgccggaagagcgcgaatggatggacaggctgatgagctgggggttggtcgataccttccgccatgcgaatccgcaaacagcagatcgtttctcatggtttgattaccgctcaaaaggttttgacgataaccgtggtctgcgcatcgacctgctgctcgccagccaaccgctggcagaatgttgcgtagaaaccggcatcgactatgaaatccgcagcatggaaaaaccgtccgatcacgcccccgtctgggcgaccttccgccgc

SEQ ID NO: 13 - DNA, 951 bp, Artificial Sequence
  P4S-EXOIII
agccccgaggacaagatcagccagctgaagcagaagatccagcagctgaagcaggagaaccagcagctggaggaggagaacagccagctggagtacggcggctctggcggcggctccggaggctctgatccaaaaaagaagagaaaggtaaaatttgtctcttttaatatcaacggcctgcgcgccagacctcaccagcttgaagccatcgtcgaaaagcaccaaccggatgtgattggcctgcaggagacaaaagttcatgacgatatgtttccgctcgaagaggtggcgaagctcggctacaacgtgttttatcacgggcagaaaggccattatggcgtggcgctgctgaccaaagagacgccgattgccgtgcgtcgcggctttcccggtgacgacgaagaggcgcagcggcggattattatggcggaaatcccctcactgctgggtaatgtcaccgtgatcaacggttacttcccgcagggtgaaagccgcgaccatccgataaaattcccggcaaaagcgcagttttatcagaatctgcaaaactacctggaaaccgaactcaaacgtgataatccggtactgattatgggcgatatgaatatcagccctacagatctggacatcggcattggcgaagaaaaccgtaagcgctggctgcgtaccggtaaatgctctttcctgccggaagagcgcgaatggatggacaggctgatgagctgggggttggtcgataccttccgccatgcgaatccgcaaacagcagatcgtttctcatggtttgattaccgctcaaaaggttttgacgataaccgtggtctgcgcatcgacctgctgctcgccagccaaccgctggcagaatgttgcgtagaaaccggcatcgactatgaaatccgcagcatggaaaaaccgtccgatcacgcccccgtctgggcgaccttccgccgc

SEQ ID NO: 14 - DNA, 951 bp, Artificial Sequence
  AP4-EXOIII
agccccgaggacgagctggccgccaacgaggaggagctgcagcagaacgagcagaagctggcccagatcaagcagaagctgcaggccatcaagtacggcggctctggcggcggctccggaggctctgatccaaaaaagaagagaaaggtaaaatttgtctcttttaatatcaacggcctgcgcgccagacctcaccagcttgaagccatcgtcgaaaagcaccaaccggatgtgattggcctgcaggagacaaaagttcatgacgatatgtttccgctcgaagaggtggcgaagctcggctacaacgtgttttatcacgggcagaaaggccattatggcgtggcgctgctgaccaaagagacgccgattgccgtgcgtcgcggctttcccggtgacgacgaagaggcgcagcggcggattattatggcggaaatcccctcactgctgggtaatgtcaccgtgatcaacggttacttcccgcagggtgaaagccgcgaccatccgataaaattcccggcaaaagcgcagttttatcagaatctgcaaaactacctggaaaccgaactcaaacgtgataatccggtactgattatgggcgatatgaatatcagccctacagatctggacatcggcattggcgaagaaaaccgtaagcgctggctgcgtaccggtaaatgctctttcctgccggaagagcgcgaatggatggacaggctgatgagctgggggttggtcgataccttccgccatgcgaatccgcaaacagcagatcgtttctcatggtttgattaccgctcaaaaggttttgacgataaccgtggtctgcgcatcgacctgctgctcgccagccaaccgctggcagaatgttgcgtagaaaccggcatcgactatgaaatccgcagcatggaaaaaccgtccgatcacgcccccgtctgggcgaccttccgccgc

SEQ ID NO: 15 - DNA, 840 bp, Artificial Sequence
  P3-TREX2
tccccggaagatgagatccagcaactggaagaagaaatcgctcagctggaacagaaaaacgcagcgctgaaagagaaaaaccaggcgctgaaatacggtggcggctctggcggcggctccggaggctctatgtctgagccacctcgggctgagacctttgtattcctggacctagaagccactgggctcccaaacatggaccctgagattgcagagatatccctttttgctgttcaccgctcttccctggagaacccagaacgggatgattctggttccttggtgctgccccgtgttctggacaagctcacactgtgcatgtgcccggagcgcccctttactgccaaggccagtgagattactggtttgagcagcgaaagcctgatgcactgcgggaaggctggtttcaatggcgctgtggtaaggacactgcagggcttcctaagccgccaggagggccccatctgccttgtggcccacaatggcttcgattatgacttcccactgctgtgcacggagctacaacgtctgggtgcccatctgccccaagacactgtctgcctggacacactgcctgcattgcggggcctggaccgtgctcacagccacggcaccagggctcaaggccgcaaaagctacagcctggccagtctcttccaccgctacttccaggctgaacccagtgctgcccattcagcagaaggtgatgtgcacaccctgcttctgatcttcctgcatcgtgctcctgagctgctcgcctgggcagatgagcaggcccgcagctgggctcatattgagcccatgtacgtgccacctgatggtccaagcctcgaagcctga

SEQ ID NO: 16 - DNA, 837 bp, Artificial Sequence
  P4-TREX2
agcccggaagataaaattgctcagctgaaacaaaaaatccaagcgctgaaacaggaaaaccagcagctggaagaggaaaacgccgcactggaatatggtggcggctctggcggcggctccggaggctcttctgagccacctcgggctgagacctttgtattcctggacctagaagccactgggctcccaaacatggaccctgagattgcagagatatccctttttgctgttcaccgctcttccctggagaacccagaacgggatgattctggttccttggtgctgccccgtgttctggacaagctcacactgtgcatgtgcccggagcgcccctttactgccaaggccagtgagattactggtttgagcagcgaaagcctgatgcactgcgggaaggctggtttcaatggcgctgtggtaaggacactgcagggcttcctaagccgccaggagggccccatctgccttgtggcccacaatggcttcgattatgacttcccactgctgtgcacggagctacaacgtctgggtgcccatctgccccaagacactgtctgcctggacacactgcctgcattgcggggcctggaccgtgctcacagccacggcaccagggctcaaggccgcaaaagctacagcctggccagtctcttccaccgctacttccaggctgaacccagtgctgcccattcagcagaaggtgatgtgcacaccctgcttctgatcttcctgcatcgtgctcctgagctgctcgcctgggcagatgagcaggcccgcagctgggctcatattgagcccatgtacgtgccacctgatggtccaagcctcgaagcctga

SEQ ID NO: 17 - DNA, 2668 bp, Artificial Sequence
  P3-EXO1
tccccggaagatgagatccagcaactggaagaagaaatcgctcagctggaacagaaaaacgcagcgctgaaagagaaaaaccaggcgctgaaatacggtggcggctctggcggcggctccggaggctctgcgatcgccatggggatacagggattgctacaatttatcaaagaagcttcagaacccatccatgtgaggaagtataaagggcaggtagtagctgtggatacatattgctggcttcacaaaggagctattgcttgtgctgaaaaactagccaaaggtgaacctactgataggtatgtaggattttgtatgaaatttgtaaatatgttactatctcatgggatcaagcctattctcgtatttgatggatgtactttaccttctaaaaaggaagtagagagatctagaagagaaagacgacaagccaatcttcttaagggaaagcaacttcttcgtgaggggaaagtctcggaagctcgagagtgtttcacccggtctatcaatatcacacatgccatggcccacaaagtaattaaagctgcccggtctcagggggtagattgcctcgtggctccctatgaagctgatgcgcagttggcctatcttaacaaagcgggaattgtgcaagccataattacagaggactcggatctcctagcttttggctgtaaaaaggtaattttaaagatggaccagtttggaaatggacttgaaattgatcaagctcggctaggaatgtgcagacagcttggggatgtattcacggaagagaagtttcgttacatgtgtattctttcaggttgtgactacctgtcatcactgcgtgggattggattagcaaaggcatgcaaagtcctaagactagccaataatccagatatagtaaaggttatcaagaaaattggacattatctcaagatgaatatcacggtaccagaggattacatcaacgggtttattcgggccaacaataccttcctctatcagctagtttttgatcccatcaaaaggaaacttattcctctgaacgcctatgaagatgatgttgatcctgaaacactaagctacgctgggcaatatgttgatgattccatagctcttcaaatagcacttggaaataaagatataaatacttttgaacagatcgatgactacaatccagacactgctatgcctgcccattcaagaagtcatagttgggatgacaaaacatgtcaaaagtcagctaatgttagcagcatttggcataggaattactctcccagaccagagtcgggtactgtttcagatgccccacaattgaaggaaaatccaagtactgtgggagtggaacgagtgattagtactaaagggttaaatctcccaaggaaatcatccattgtgaaaagaccaagaagtgcagagctgtcagaagatgacctgttgagtcagtattctctttcatttacgaagaagaccaagaaaaatagctctgaaggcaataaatcattgagcttttctgaagtgtttgtgcctgacctggtaaatggacctactaacaaaaagagtgtaagcactccacctaggacgagaaataaatttgcaacatttttacaaaggaaaaatgaagaaagtggtgcagttgtggttccagggaccagaagcaggtttttttgcagttcagattctactgactgtgtatcaaacaaagtgagcatccagcctctggatgaaactgctgtcacagataaagagaacaatctgcatgaatcagagtatggagaccaagaaggcaagagactggttgacacagatgtagcacgtaattcaagtgatgacattccgaataatcatattccaggtgatcatattccagacaaggcaacagtgtttacagatgaagagtcctactcttttgagagcagcaaatttacaaggaccatttcaccacccactttgggaacactaagaagttgttttagttggtctggaggtcttggagatttttcaagaacgccgagcccctctccaagcacagcattgcagcagttccgaagaaagagcgattcccccacctctttgcctgagaataatatgtctgatgtgtcgcagttaaagagcgaggagtccagtgacgatgagtctcatcccttacgagaaggggcatgttcttcacagtcccaggaaagtggagaattctcactgcagagttcaaatgcatcaaagctttctcagtgctctagtaaggactctgattcagaggaatctgattgcaatattaagttacttgacagtcaaagtgaccagacctccaagctatgtttatctcatttctcaaaaaaagacacacctctaaggaacaaggttcctgggctatataagtccagttctgcagactctctttctacaaccaagatcaaacctctaggacctgccagagccagtgggctgagcaagaagccggcaagcatccagaagagaaagcatcataatgccgagaacaagccggggttacagatcaaactcaatgagctctggaaaaactttggatttaaaaaagattctgaaaagcttcctccttgtaagaaacccctgtccccagtcagagataacatccaactaactccagaagcggaagaggatatatttaacaaacctgaatgtggccgtgttcaaagagcaa

SEQ ID NO: 18 - DNA, 2668 bp, Artificial Sequence
  P4-EXO1
agcccggaagataaaattgctcagctgaaacaaaaaatccaagcgctgaaacaggaaaaccagcagctggaagaggaaaacgccgcactggaatatggtggcggctctggcggcggctccggaggctctgcgatcgccatggggatacagggattgctacaatttatcaaagaagcttcagaacccatccatgtgaggaagtataaagggcaggtagtagctgtggatacatattgctggcttcacaaaggagctattgcttgtgctgaaaaactagccaaaggtgaacctactgataggtatgtaggattttgtatgaaatttgtaaatatgttactatctcatgggatcaagcctattctcgtatttgatggatgtactttaccttctaaaaaggaagtagagagatctagaagagaaagacgacaagccaatcttcttaagggaaagcaacttcttcgtgaggggaaagtctcggaagctcgagagtgtttcacccggtctatcaatatcacacatgccatggcccacaaagtaattaaagctgcccggtctcagggggtagattgcctcgtggctccctatgaagctgatgcgcagttggcctatcttaacaaagcgggaattgtgcaagccataattacagaggactcggatctcctagcttttggctgtaaaaaggtaattttaaagatggaccagtttggaaatggacttgaaattgatcaagctcggctaggaatgtgcagacagcttggggatgtattcacggaagagaagtttcgttacatgtgtattctttcaggttgtgactacctgtcatcactgcgtgggattggattagcaaaggcatgcaaagtcctaagactagccaataatccagatatagtaaaggttatcaagaaaattggacattatctcaagatgaatatcacggtaccagaggattacatcaacgggtttattcgggccaacaataccttcctctatcagctagtttttgatcccatcaaaaggaaacttattcctctgaacgcctatgaagatgatgttgatcctgaaacactaagctacgctgggcaatatgttgatgattccatagctcttcaaatagcacttggaaataaagatataaatacttttgaacagatcgatgactacaatccagacactgctatgcctgcccattcaagaagtcatagttgggatgacaaaacatgtcaaaagtcagctaatgttagcagcatttggcataggaattactctcccagaccagagtcgggtactgtttcagatgccccacaattgaaggaaaatccaagtactgtgggagtggaacgagtgattagtactaaagggttaaatctcccaaggaaatcatccattgtgaaaagaccaagaagtgcagagctgtcagaagatgacctgttgagtcagtattctctttcatttacgaagaagaccaagaaaaatagctctgaaggcaataaatcattgagcttttctgaagtgtttgtgcctgacctggtaaatggacctactaacaaaaagagtgtaagcactccacctaggacgagaaataaatttgcaacatttttacaaaggaaaaatgaagaaagtggtgcagttgtggttccagggaccagaagcaggtttttttgcagttcagattctactgactgtgtatcaaacaaagtgagcatccagcctctggatgaaactgctgtcacagataaagagaacaatctgcatgaatcagagtatggagaccaagaaggcaagagactggttgacacagatgtagcacgtaattcaagtgatgacattccgaataatcatattccaggtgatcatattccagacaaggcaacagtgtttacagatgaagagtcctactcttttgagagcagcaaatttacaaggaccatttcaccacccactttgggaacactaagaagttgttttagttggtctggaggtcttggagatttttcaagaacgccgagcccctctccaagcacagcattgcagcagttccgaagaaagagcgattcccccacctctttgcctgagaataatatgtctgatgtgtcgcagttaaagagcgaggagtccagtgacgatgagtctcatcccttacgagaaggggcatgttcttcacagtcccaggaaagtggagaattctcactgcagagttcaaatgcatcaaagctttctcagtgctctagtaaggactctgattcagaggaatctgattgcaatattaagttacttgacagtcaaagtgaccagacctccaagctatgtttatctcatttctcaaaaaaagacacacctctaaggaacaaggttcctgggctatataagtccagttctgcagactctctttctacaaccaagatcaaacctctaggacctgccagagccagtgggctgagcaagaagccggcaagcatccagaagagaaagcatcataatgccgagaacaagccggggttacagatcaaactcaatgagctctggaaaaactttggatttaaaaaagattctgaaaagcttcctccttgtaagaaacccctgtccccagtcagagataacatccaactaactccagaagcggaagaggatatatttaacaaacctgaatgtggccgtgttcaaagagcaa

SEQ ID NO: 19 - DNA, 20 bp, artificial sequence
  targeting sequence in eGFP genomic region
ggcgagggcgatgccaccta

SEQ ID NO: 20 - DNA, 20 bp, artificial sequence
  human EMX1 gene targeting sequence
gagtccgagcagaagaagaa

SEQ ID NO: 21 - DNA, 20 bp, artificial sequence
  human VEGF gene targeting sequence
ggtgagtgagtgtgtgcgtg

SEQ ID NO: 22 - DNA, 20 bp, artificial sequence
  human MYD88 gene targeting sequence
ggctgagaagcctttacagg

SEQ ID NO: 23 - DNA, 20 bp, artificial sequence
  human ANKRD52 gene targeting sequence
actgtaaaggctgctctccc

SEQ ID NO: 24 - DNA, 20 bp, artificial sequence
  human FUT9 gene target sequence
tgcagaggagcctttacatg

SEQ ID NO: 25 - DNA, 20 bp, artificial sequence
  human PSKH2 gene targeting sequence
gccagacaaggctttacagg

SEQ ID NO: 26 - DNA, 20 bp, artificial sequence
  human BCR-ABL fusion gene targeting sequence
gacctgtcttttagacaggc

SEQ ID NO: 27 - DNA, 40 bp, artificial sequence
  equivalent Cas9 protein expression - pcDNA3
ggaggctgagaagcctttacaggtggccgctgtagacagc

SEQ ID NO: 28 - DNA, 31 bp, artificial sequence
  equivalent Cas9 protein expression - Cas9
ggaggctgagaaggtggccgctgtagacagc

SEQ ID NO: 29 - DNA, 26 bp, artificial sequence
  equivalent Cas9 protein expression - Cas9+EXO3
ggaggcaggtggccgctgtagacagc